European Patent Specification EP 3 463 481 B1, published April 30, 2025. Title: BIODEGRADABLE DENDRITIC STRUCTURE, METHODS AND USES THEREOF. Applicant: INSTITUTO NACIONAL DE ENGENHARIA BIOMÉDICA. The sequence listing filed with the application follows.

SEQUENCE LISTING (1 sequence)

SEQ ID NO: 1 - RNA, 25 nt, synthetic construct
gcugacccugaaguucaucugcacc